European Patent Specification EP 3 795 181 B1, published August 6, 2025. Title: TREATMENT OF AMD USING AAV2 VARIANT WITH AFLIBERCEPT. Applicant: ADVERUM BIOTECHNOLOGIES, INC. Application PCT/US2017/038003. The sequence listing filed with the application follows.

SEQUENCE LISTING (11 sequences)

SEQ ID NO: 1 - protein, 431 aa, Artificial Sequence
  Description of Artificial Sequence: Synthetic polypeptide
SDTGRPFVEMYSEIPEIIHMTEGRELVIPCRVTSPNITVTLKKFPLDTLIPDGKRIIWDSRKGFIISNATYKEIGLLTCEATVNGHLYKTNYLTHRQTNTIIDVVLSPSHGIELSVGEKLVLNCTARTELNVGIDFNWEYPSSKHQHKKLVNRDLKTQSGSEMKKFLSTLTIDGVTRSDQGLYTCAASSGLMTKKNSTFVRVHEKDKTHTCPPCPAPELLGGPSVFLFPPKPKDTLMISRTPEVTCVVVDVSHEDPEVKFNWYVDGVEVHNAKTKPREEQYNSTYRVVSVLTVLHQDWLNGKEYKCKVSNKALPAPIEKTISKAKGQPREPQVYTLPPSRDELTKNQVSLTCLVKGFYPSDIAVEWESNGQPENNYKTTPPVLDSDGSFFLYSKLTVDKSRWQQGNVFSCSVMHEALHNHYTQKSLSLSPG

SEQ ID NO: 2 - DNA, 1377 bp, Artificial Sequence
  Description of Artificial Sequence: Synthetic polynucleotide
atggtcagctactgggacaccggggtcctgctgtgcgcgctgctcagctgtctgcttctcacaggatctagttccggaagtgataccggtagacctttcgtagagatgtacagtgaaatccccgaaattatacacatgactgaaggaagggagctcgtcattccctgccgggttacgtcacctaacatcactgttactttaaaaaagtttccacttgacactttgatccctgatggaaaacgcataatctgggacagtagaaagggcttcatcatatcaaatgcaacgtacaaagaaatagggcttctgacctgtgaagcaacagtcaatgggcatttgtataagacaaactatctcacacatcgacaaaccaatacaatcatagatgtggttctgagtccgtctcatggaattgaactatctgttggagaaaagcttgtcttaaattgtacagcaagaactgaactaaatgtggggattgacttcaactgggaatacccttcttcgaagcatcagcataagaaacttgtaaaccgagacctaaaaacccagtctgggagtgagatgaagaaatttttgagcaccttaactatagatggtgtaacccggagtgaccaaggattgtacacctgtgcagcatccagtgggctgatgaccaagaagaacagcacatttgtcagggtccatgaaaaggacaaaactcacacatgcccaccgtgcccagcacctgaactcctggggggaccgtcagtcttcctcttccccccaaaacccaaggacaccctcatgatctcccggacccctgaggtcacatgcgtggtggtggacgtgagccacgaagaccctgaggtcaagttcaactggtacgtggacggcgtggaggtgcataatgccaagacaaagccgcgggaggagcagtacaacagcacgtaccgtgtggtcagcgtcctcaccgtcctgcaccaggactggctgaatggcaaggagtacaagtgcaaggtctccaacaaagccctcccagcccccatcgagaaaaccatctccaaagccaaagggcagccccgagaaccacaggtgtacaccctgcccccatcccgggatgagctgaccaagaaccaggtcagcctgacctgcctggtcaaaggcttctatcccagcgacatcgccgtggagtgggagagcaatgggcagccggagaacaactacaagaccacgcctcccgtgctggactccgacggctccttcttcctctacagcaagctcaccgtggacaagagcaggtggcagcaggggaacgtcttctcatgctccgtgatgcatgaggctctgcacaaccactacacgcagaagagcctctccctgtctccgggtaaatga

SEQ ID NO: 3 - DNA, 2064 bp, Homo sapiens
atggtcagctactgggacaccggggtcctgctgtgcgcgctgctcagctgtctgcttctcacaggatctagttcaggttcaaaattaaaagatcctgaactgagtttaaaaggcacccagcacatcatgcaagcaggccagacactgcatctccaatgcaggggggaagcagcccataaatggtctttgcctgaaatggtgagtaaggaaagcgaaaggctgagcataactaaatctgcctgtggaagaaatggcaaacaattctgcagtactttaaccttgaacacagctcaagcaaaccacactggcttctacagctgcaaatatctagctgtacctacttcaaagaagaaggaaacagaatctgcaatctatatatttattagtgatacaggtagacctttcgtagagatgtacagtgaaatccccgaaattatacacatgactgaaggaagggagctcgtcattccctgccgggttacgtcacctaacatcactgttactttaaaaaagtttccacttgacactttgatccctgatggaaaacgcataatctgggacagtagaaagggcttcatcatatcaaatgcaacgtacaaagaaatagggcttctgacctgtgaagcaacagtcaatgggcatttgtataagacaaactatctcacacatcgacaaaccaatacaatcatagatgtccaaataagcacaccacgcccagtcaaattacttagaggccatactcttgtcctcaattgtactgctaccactcccttgaacacgagagttcaaatgacctggagttaccctgatgaaaaaaataagagagcttccgtaaggcgacgaattgaccaaagcaattcccatgccaacatattctacagtgttcttactattgacaaaatgcagaacaaagacaaaggactttatacttgtcgtgtaaggagtggaccatcattcaaatctgttaacacctcagtgcatatatatgataaagcattcatcactgtgaaacatcgaaaacagcaggtgcttgaaaccgtagctggcaagcggtcttaccggctctctatgaaagtgaaggcatttccctcgccggaagttgtatggttaaaagatgggttacctgcgactgagaaatctgctcgctatttgactcgtggctactcgttaattatcaaggacgtaactgaagaggatgcagggaattatacaatcttgctgagcataaaacagtcaaatgtgtttaaaaacctcactgccactctaattgtcaatgtgaaaccccagatttacgaaaaggccgtgtcatcgtttccagacccggctctctacccactgggcagcagacaaatcctgacttgtaccgcatatggtatccctcaacctacaatcaagtggttctggcacccctgtaaccataatcattccgaagcaaggtgtgacttttgttccaataatgaagagtcctttatcctggatgctgacagcaacatgggaaacagaattgagagcatcactcagcgcatggcaataatagaaggaaagaataagatggctagcaccttggttgtggctgactctagaatttctggaatctacatttgcatagcttccaataaagttgggactgtgggaagaaacataagcttttatatcacagatgtgccaaatgggtttcatgttaacttggaaaaaatgccgacggaaggagaggacctgaaactgtcttgcacagttaacaagttcttatacagagacgttacttggattttactgcggacagttaataacagaacaatgcactacagtattagcaagcaaaaaatggccatcactaaggagcactccatcactcttaatcttaccatcatgaatgtttccctgcaagattcaggcacctatgcctgcagagccaggaatgtatacacaggggaagaaatcctccagaagaaagaaattacaatcagaggtgagcactgcaacaaaaaggctgttttctctcggatctccaaatttaaaagcacaaggaatgattgtaccacacaaagtaatgtaaaacattaa

SEQ ID NO: 4 - protein, 7 aa, Artificial Sequence
  Description of Artificial Sequence: Synthetic peptide
LGETTRP

SEQ ID NO: 5 - protein, 7 aa, Artificial Sequence
  Description of Artificial Sequence: Synthetic peptide
NETITRP

SEQ ID NO: 6 - protein, 7 aa, Artificial Sequence
  Description of Artificial Sequence: Synthetic peptide
KAGQANN

SEQ ID NO: 7 - protein, 7 aa, Artificial Sequence
  Description of Artificial Sequence: Synthetic peptide
KDPKTTN

SEQ ID NO: 8 - protein, 7 aa, Artificial Sequence
  Description of Artificial Sequence: Synthetic peptide
KDTDTTR

SEQ ID NO: 9 - protein, 7 aa, Artificial Sequence
  Description of Artificial Sequence: Synthetic peptide
RAGGSVG

SEQ ID NO: 10 - protein, 7 aa, Artificial Sequence
  Description of Artificial Sequence: Synthetic peptide
AVDTTKF

SEQ ID NO: 11 - protein, 7 aa, Artificial Sequence
  Description of Artificial Sequence: Synthetic peptide
STGKVPN